European Patent Application EP 4 556 493 A1, published May 21, 2025. Title: CYTOKINE FUSION PROTEIN. Applicant: 주식회사 지뉴브. Application KR. The sequence listing filed with the application follows.

SEQUENCE LISTING (61 sequences)

SEQ ID NO: 1 - protein, 133 aa, Homo sapiens [sequence omitted]

SEQ ID NO: 2 - protein, 133 aa, Homo sapiens
APTSSSTKKTQLQLEHLLLDLQMILNGINNYKNPKLTRMLTFKFYMPKKATELKHLQCLEEELKPLEEVLNLAQSKNFHLRPRDLISNINVIVLELKGSETTFMCEYADETATIVEFLNRWITFSQSIISTLT

SEQ ID NO: 3 - protein, 251 aa, Homo sapiens
ELCDDDPPEIPHATFKAMAYKEGTMLNCECKRGFRRIKSGSLYMLCTGNSSHSSWDNQCQCTSSATRNTTKQVTPQPEEQKERKTTEMQSPMQPVDQASLPGHCREPPPWENEATERIYHFVVGQMVYYQCVQGYRALHRGPAESVCKMTHGKTRWTQPQLICTGEMETSQFPGEEKPQASPEGRPESETSCLVTTTDFQIQTEMAATMETSIFTTEYQVAVAGCVFLLISVLLLSGLTWQRRQRKSRRTI

SEQ ID NO: 4 - protein, 219 aa, Homo sapiens
ELCDDDPPEIPHATFKAMAYKEGTMLNCECKRGFRRIKSGSLYMLCTGNSSHSSWDNQCQCTSSATRNTTKQVTPQPEEQKERKTTEMQSPMQPVDQASLPGHCREPPPWENEATERIYHFVVGQMVYYQCVQGYRALHRGPAESVCKMTHGKTRWTQPQLICTGEMETSQFPGEEKPQASPEGRPESETSCLVTTTDFQIQTEMAATMETSIFTTEYQ

SEQ ID NO: 5 - protein, 165 aa, Homo sapiens
ELCDDDPPEIPHATFKAMAYKEGTMLNCECKRGFRRIKSGSIYMLCTGNSSHSSWDNQCQCTSSATRNTTKQVTPQPEEQKERKTTEMQSPMQPVDQASLPGHCREPPPWENEATERIYHFVVGQMVYYQCVQGYRALHRGPAESVCKMTHGKTRWTQPQLICTG

SEQ ID NO: 6 - protein, 114 aa, Homo sapiens
NWVNVISDLKKIEDLIQSMHIDATLYTESDVHPSCKVTAMKCFLLELQVISLESGDASIHDTVENLIILANNSLSSNGNVTESGCKECEELEEKNIKEFLQSFVHIVQMFINTS

SEQ ID NO: 7 - protein, 237 aa, Homo sapiens
ITCPPPMSVEHADIWVKSYSLYSRERYICNSGFKRKAGTSSLTECVLNKATNVAHWTTPSLKCIRDPALVHQRPAPPSTVTTAGVTPQPESLSPSGKEPAASSPSSNNTAATTAAIVPGSQLMPSKSPSTGTTEISSHESSHGTPSQTTAKNWELTASASHQPPGVYPQGHSDTTVAISTSTVLLCGLSAVSLLACYLKSRQTPPLASVEMEAMEALPVTWGTSSRDEDLENCSHHL

SEQ ID NO: 8 - protein, 175 aa, Homo sapiens
ITCPPPMSVEHADIWVKSYSLYSRERYICNSGFKRKAGTSSLTECVLNKATNVAHWTTPSLKCIRDPALVHQRPAPPSTVTTAGVTPQPESLSPSGKEPAASSPSSNNTAATTAAIVPGSQLMPSKSPSTGTTEISSHESSHGTPSQTTAKNWELTASASHQPPGVYPQGHSDTT

SEQ ID NO: 9 - protein, 5 aa, synthetic construct
GYWMH

SEQ ID NO: 10 - protein, 17 aa, synthetic construct
MIHPNSDTTTYNEKFKN

SEQ ID NO: 11 - protein, 17 aa, synthetic construct
MIHPNSDTTVYNEKFKN

SEQ ID NO: 12 - protein, 17 aa, synthetic construct
MIHPNSDTTIYNEKFKN

SEQ ID NO: 13 - protein, 17 aa, synthetic construct
MIHPNSDTTTYNWKFKN

SEQ ID NO: 14 - protein, 17 aa, synthetic construct
MIHPNSDTTVYNWKFKN

SEQ ID NO: 15 - protein, 17 aa, synthetic construct
MIHPNSDTTIYNWKFKN

SEQ ID NO: 16 - protein, 9 aa, synthetic construct
TDQAAWFAF

SEQ ID NO: 17 - protein, 9 aa, synthetic construct
TDQEAWFAF

SEQ ID NO: 18 - protein, 9 aa, synthetic construct
TDQAAWAAF

SEQ ID NO: 19 - protein, 9 aa, synthetic construct
TDQAAWMAF

SEQ ID NO: 20 - protein, 9 aa, synthetic construct
TDQAAWHAF

SEQ ID NO: 21 - protein, 9 aa, synthetic construct
TDQAAWFGF

SEQ ID NO: 22 - protein, 9 aa, synthetic construct
TDQEAWAAF

SEQ ID NO: 23 - protein, 9 aa, synthetic construct
TDQEAWMAF

SEQ ID NO: 24 - protein, 9 aa, synthetic construct
TDQEAWHAF

SEQ ID NO: 25 - protein, 9 aa, synthetic construct
TDQEAWFGF

SEQ ID NO: 26 - protein, 9 aa, synthetic construct
TDQAAWAGF

SEQ ID NO: 27 - protein, 9 aa, synthetic construct
TDQAAWMGF

SEQ ID NO: 28 - protein, 9 aa, synthetic construct
TDQAAWHGF

SEQ ID NO: 29 - protein, 9 aa, synthetic construct
TDQEAWAGF

SEQ ID NO: 30 - protein, 9 aa, synthetic construct
TDQEAWMGF

SEQ ID NO: 31 - protein, 9 aa, synthetic construct
TDQEAWHGF

SEQ ID NO: 32 - protein, 16 aa, synthetic construct
RSSQNIVHSNGDTYLE

SEQ ID NO: 33 - protein, 16 aa, synthetic construct
RSSQNIVHSQGDTYLE

SEQ ID NO: 34 - protein, 16 aa, synthetic construct
RSSQNIVRSNGDTYLE

SEQ ID NO: 35 - protein, 16 aa, synthetic construct
RSSQNIVRSQGDTYLE

SEQ ID NO: 36 - protein, 7 aa, synthetic construct
KVSKRFS

SEQ ID NO: 37 - protein, 9 aa, synthetic construct
FQGSHVPWT

SEQ ID NO: 38 - protein, 118 aa, synthetic construct
EVQLQQSGAELVKPGASVKLSCKASGYTFTGYWMHWVKQRPGQGLEWIGMIHPNSDTTTYNEKFKNRATLTVDKSSGTAYMQLSSLTSEDSAVYYCTGTDQAAWFAFWGQGTLVTVSA

SEQ ID NO: 39 - protein, 112 aa, synthetic construct
DIVLTQTPLSLPVSLGDQASISCRSSQNIVHSNGDTYLEWYLQKPGQSPKLLIYKVSKRFSGVPDRFSGSGSGTDFTLKISRVEAEDLGVYYCFQGSHVPWTFGGGTKLEIK

SEQ ID NO: 40 - protein, 118 aa, synthetic construct
QVQLVQSGAEVKKPGASVKVSCKASGYTFTGYWMHWVRQAPGQGLEWMGMIHPNSDTTTYNEKFKNRVTMTRDTSISTAYMELSRLRSDDTAVYYCAGTDQAAWFAFWGQGTTVTVSS

SEQ ID NO: 41 - protein, 112 aa, synthetic construct
DIVMTQTPLSLSVTPGQPASISCRSSQNIVHSNGDTYLEWYLQKPGQSPKLLIYKVSKRFSGVPDRFSGSGSGTDFTLKISRVEAEDVGVYYCFQGSHVPWTFGGGTKVEIK

SEQ ID NO: 42 - protein, 118 aa, synthetic construct
QVQLVQSGAEVKKPGASVKVSCKASGYTFTGYWMHWVRQAPGQGLEWIGMIHPNSDTTTYNEKFKNRVTMTRDTSISTAYMELSRLRSDDTAVYYCTGTDQAAWFAFWGQGTTVTVSS

SEQ ID NO: 43 - protein, 112 aa, synthetic construct
DIVMTQTPLSLSVTPGQPASISCRSSQNIVHSNGDTYLEWYLQKPGQSPQLLIYKVSKRFSGVPDRFSGSGSGTDFTLKISRVEAEDVGVYYCFQGSHVPWTFGGGTKVEIK

SEQ ID NO: 44 - protein, 118 aa, synthetic construct
QVQLVQSGAEVKKPGASVKVSCKASGYTFTGYWMHWVRQAPGQGLEWIGMIHPNSDTTTYNEKFKNRVTMTRDTSISTAYMELSRLRSDDTAVYYCAGTDQAAWFAFWGQGTTVTVSS

SEQ ID NO: 45 - protein, 112 aa, synthetic construct
DIVMTQTPLSLSVTPGQPASISCRSSQNIVHSQGDTYLEWYLQKPGQSPQLLIYKVSKRFSGVPDRFSGSGSGTDFTLKISRVEAEDVGVYYCFQGSHVPWTFGGGTKVEIK

SEQ ID NO: 46 - protein, 327 aa, Homo sapiens
ASTKGPSVFPLAPCSRSTSESTAALGCLVKDYFPEPVTVSWNSGALTSGVHTFPAVLQSSGLYSLSSVVTVPSSSLGTKTYTCNVDHKPSNTKVDKRVESKYGPPCPPCPAPEFLGGPSVFLFPPKPKDTLMISRTPEVTCVVVDVSQEDPEVQFNWYVDGVEVHNAKTKPREEQFNSTYRVVSVLTVLHQDWLNGKEYKCKVSNKGLPSSIEKTISKAKGQPREPQVYTLPPSQEEMTKNQVSLTCLVKGFYPSDIAVEWESNGQPENNYKTTPPVLDSDGSFFLYSRLTVDKSRWQEGNVFSCSVMHEALHNHYTQKSLSLSPGK

SEQ ID NO: 47 - protein, 107 aa, Homo sapiens [sequence omitted]

SEQ ID NO: 48 - protein, 288 aa, Homo sapiens
MQIPQAPWPVVWAVLQLGWRPGWFLDSPDRPWNPPTFSPALLVVTEGDNATFTCSFSNTSESFVLNWYRMSPSNQTDKLAAFPEDRSQPGQDCRFRVTQLPNGRDFHMSVVRARRNDSGTYLCGAISLAPKAQIKESLRAELRVTERRAEVPTAHPSPSPRPAGQFQTLVVGVVGGLLGSLVLLVWVLAVICSRAARGTIGARRTGQPLKEDPSAVPVFSVDYGELDFQWREKTPEPPVPCVPEQTEYATIVFPSGMGTSSPARRGSADGPRSAQPLRPEDGHCSWPL

SEQ ID NO: 49 - protein, 229 aa, synthetic construct
ESKYGPPCPPCPAPEFLGGPSVFLFPPKPKDTLMISRTPEVTCVVVDVSQEDPEVQFNWYVDGVEVHNAKTKPREEQFNSTYRVVSVLTVLHQDWLNGKEYKCKVSNKGLPSSIEKTISKAKGQPREPRVYTLPPSQEEMTKNQVSLWCLVKGFYPSDIAVEWESNGQPENNYKTTPPVLDSDGSFFLYSRLTVDKSRWQEGNVFSCSVMHEALHNHYTQKSLSLSPGK

SEQ ID NO: 50 - protein, 229 aa, synthetic construct
ESKYGPPCPPCPAPEFLGGPSVFLFPPKPKDTLMISRTPEVTCVVVDVSQEDPEVQFNWYVDGVEVHNAKTKPREEQFNSTYRVVSVLTVLHQDWLNGKEYKCKVSNKGLPSSIEKTISKAKGQPREPQVYTLPPSQEEMTENQVSLSCAVKGFYPSDIAVEWESNGQPENNYKTTPPVLDSDGSFFLVSRLTVDKSRWQEGNVFSCSVMHEALHNHYTQKSLSLSPGK

SEQ ID NO: 51 - protein, 219 aa, synthetic construct
DIVMTQTPLSLSVTPGQPASISCRSSQNIVHSQGDTYLEWYLQKPGQSPQLLIYKVSKRFSGVPDRFSGSGSGTDFTLKISRVEAEDVGVYYCFQGSHVPWTFGGGTKVEIKRTVAAPSVFIFPPSDEQLKSGTASVVCLLNNFYPREAKVQWKVDNALQSGNSQESVTEQDSKDSTYSLSSTLTLSKADYEKHKVYACEVTHQGLSSPVTKSFNRGEC

SEQ ID NO: 52 - protein, 216 aa, synthetic construct
QVQLVQSGAEVKKPGASVKVSCKASGYTFTGYWMHWVRQAPGQGLEWIGMIHPNSDTTTYNEKFKNRVTMTRDTSISTAYMELSRLRSDDTAVYYCAGTDQAAWFAFWGQGTTVTVSSASTKGPSVFPLAPCSRSTSESTAALGCLVKDYFPEPVTVSWNSGALTSGVHTFPAVLQSSGLYSLSSVVTVPSSSLGTKTYTCNVDHKPSNTKVDKRV

SEQ ID NO: 53 - DNA, 39 bp, synthetic construct
  source 1..39: mol_type = other DNA
ccctctcccccggcaagtcaggaggtggatctggtggag

SEQ ID NO: 54 - DNA, 42 bp, synthetic construct
  source 1..42: mol_type = other DNA
gcccgaattcggcggccgctttatcaggtcagcgtagagatg

SEQ ID NO: 55 - DNA, 99 bp, synthetic construct
  source 1..99: mol_type = other DNA
tctccctgtctccgggtaaaggaggtggaggttctggtggaggtggatctggtggaggaggttctggtggaggtggatctgagctgtgtgatgatgatc

SEQ ID NO: 56 - DNA, 44 bp, synthetic construct
  source 1..44: mol_type = other DNA
gtcattggggaaacctgctcctaggtttagccggtacagatcag

SEQ ID NO: 57 - protein, 593 aa, synthetic construct
QVQLVQSGAEVKKPGASVKVSCKASGYTFTGYWMHWVRQAPGQGLEWIGMIHPNSDTTTYNEKFKNRVTMTRDTSISTAYMELSRLRSDDTAVYYCAGTDQAAWFAFWGQGTTVTVSSASTKGPSVFPLAPCSRSTSESTAALGCLVKDYFPEPVTVSWNSGALTSGVHTFPAVLQSSGLYSLSSVVTVPSSSLGTKTYTCNVDHKPSNTKVDKRVESKYGPPCPPCPAPEFLGGPSVFLFPPKPKDTLMISRTPEVTCVVVDVSQEDPEVQFNWYVDGVEVHNAKTKPREEQFNSTYRVVSVLTVLHQDWLNGKEYKCKVSNKGLPSSIEKTISKAKGQPREPRVYTLPPSQEEMTKNQVSLWCLVKGFYPSDIAVEWESNGQPENNYKTTPPVLDSDGSFFLYSRLTVDKSRWQEGNVFSCSVMHEALHNHYTQKSLSLSPGKSGGGSGGGSGGGSGGAPTSSSTKKTQLQLEHLLLDLQMILNGINNYKNPKLTRMLTFKFYMPKKATELKHLQCLEEELKPLEEVLNLAQSKNFHLRPRDLISNINVIVLELKGSETTFMCEYADETATIVEFLNRWITFSQSIISTLT

SEQ ID NO: 58 - protein, 630 aa, synthetic construct
QVQLVQSGAEVKKPGASVKVSCKASGYTFTGYWMHWVRQAPGQGLEWIGMIHPNSDTTTYNEKFKNRVTMTRDTSISTAYMELSRLRSDDTAVYYCAGTDQAAWFAFWGQGTTVTVSSASTKGPSVFPLAPCSRSTSESTAALGCLVKDYFPEPVTVSWNSGALTSGVHTFPAVLQSSGLYSLSSVVTVPSSSLGTKTYTCNVDHKPSNTKVDKRVESKYGPPCPPCPAPEFLGGPSVFLFPPKPKDTLMISRTPEVTCVVVDVSQEDPEVQFNWYVDGVEVHNAKTKPREEQFNSTYRVVSVLTVLHQDWLNGKEYKCKVSNKGLPSSIEKTISKAKGQPREPQVYTLPPSQEEMTENQVSLSCAVKGFYPSDIAVEWESNGQPENNYKTTPPVLDSDGSFFLVSRLTVDKSRWQEGNVFSCSVMHEALHNHYTQKSLSLSPGKGGGGSGGGGSGGGGSGGGGSELCDDDPPEIPHATFKAMAYKEGTMLNCECKRGFRRIKSGSIYMLCTGNSSHSSWDNQCQCTSSATRNTTKQVTPQPEEQKERKTTEMQSPMQPVDQASLPGHCREPPPWENEATERIYHFVVGQMVYYQCVQGYRALHRGPAESVCKMTHGKTRWTQPQLICTG

SEQ ID NO: 59 - protein, 375 aa, synthetic construct
KYGPPCPPCPAPEFLGGPSVFLFPPKPKDTLMISRTPEVTCVVVDVSQEDPEVQFNWYVDGVEVHNAKTKPREEQFNSTYRVVSVLTVLHQDWLNGKEYKCKVSNKGLPSSIEKTISKAKGQPREPRVYTLPPSQEEMTKNQVSLWCLVKGFYPSDIAVEWESNGQPENNYKTTPPVLDSDGSFFLYSRLTVDKSRWQEGNVFSCSVMHEALHNHYTQKSLSLSPGKSGGGSGGGSGGGSGGAPTSSSTKKTQLQLEHLLLDLQMILNGINNYKNPKLTRMLTFKFYMPKKATELKHLQCLEEELKPLEEVLNLAQSKNFHLRPRDLISNINVIVLELKGSETTFMCEYADETATIVEFLNRWITFSQSIISTLT

SEQ ID NO: 60 - protein, 445 aa, synthetic construct
QVQLVQSGAEVKKPGASVKVSCKASGYTFTGYWMHWVRQAPGQGLEWIGMIHPNSDTTTYNEKFKNRVTMTRDTSISTAYMELSRLRSDDTAVYYCAGTDQAAWFAFWGQGTTVTVSSASTKGPSVFPLAPCSRSTSESTAALGCLVKDYFPEPVTVSWNSGALTSGVHTFPAVLQSSGLYSLSSVVTVPSSSLGTKTYTCNVDHKPSNTKVDKRVESKYGPPCPPCPAPEFLGGPSVFLFPPKPKDTLMISRTPEVTCVVVDVSQEDPEVQFNWYVDGVEVHNAKTKPREEQFNSTYRVVSVLTVLHQDWLNGKEYKCKVSNKGLPSSIEKTISKAKGQPREPRVYTLPPSQEEMTKNQVSLWCLVKGFYPSDIAVEWESNGQPENNYKTTPPVLDSDGSFFLYSRLTVDKSRWQEGNVFSCSVMHEALHNHYTQKSLSLSPGK

SEQ ID NO: 61 - protein, 630 aa, synthetic construct
QVQLVQSGAEVKKPGASVKVSCKASGYTFTGYWMHWVRQAPGQGLEWIGMIHPNSDTTTYNEKFKNRVTMTRDTSISTAYMELSRLRSDDTAVYYCAGTDQAAWFAFWGQGTTVTVSSASTKGPSVFPLAPCSRSTSESTAALGCLVKDYFPEPVTVSWNSGALTSGVHTFPAVLQSSGLYSLSSVVTVPSSSLGTKTYTCNVDHKPSNTKVDKRVESKYGPPCPPCPAPEFLGGPSVFLFPPKPKDTLMISRTPEVTCVVVDVSQEDPEVQFNWYVDGVEVHNAKTKPREEQFNSTYRVVSVLTVLHQDWLNGKEYKCKVSNKGLPSSIEKTISKAKGQPREPQVYTLPPSQEEMTKNQVSLTCLVKGFYPSDIAVEWESNGQPENNYKTTPPVLDSDGSFFLYSRLTVDKSRWQEGNVFSCSVMHEALHNHYTQKSLSLSPGKGGGGSGGGGSGGGGSGGGGSELCDDDPPEIPHATFKAMAYKEGTMLNCECKRGFRRIKSGSIYMLCTGNSSHSSWDNQCQCTSSATRNTTKQVTPQPEEQKERKTTEMQSPMQPVDQASLPGHCREPPPWENEATERIYHFVVGQMVYYQCVQGYRALHRGPAESVCKMTHGKTRWTQPQLICTG